European Patent Specification EP 3 988 119 B1, published October 8, 2025. Title: A PHARMACEUTICAL COMPOSITION FOR ORAL ADMINISTRATION FOR ERADICATING HELICOBACTER PYLORI COMPRISING A COMPLEX OF NON-ABSORBABLE ANTIBIOTIC AND CLAY MINERAL. Applicant: KOREA INSTITUTE OF GEOSCIENCE AND MINERAL RESOURCES. The sequence listing filed with the application follows.

SEQUENCE LISTING (4 sequences)

SEQ ID NO: 1 - DNA, 20 bp, Artificial Sequence
  sense primer for amplification of ureA and ureC specific for H. pylori.
tgatgctccactacgctgga

SEQ ID NO: 2 - DNA, 20 bp, Artificial Sequence
  antisense primer for amplification of ureA and ureC specific for H. pylori.
gggtatgcacggttacgagt

SEQ ID NO: 3 - DNA, 19 bp, Artificial Sequence
  sense primer for amplification of GAPDH
tggggtgatgctggtgctg

SEQ ID NO: 4 - DNA, 21 bp, Artificial Sequence
  antisense primer for amplification of GAPDH
ggtttctccaggcggcatgtc